European Patent Application EP 4 295 863 A1, published December 27, 2023. Title: Anti-inflammatory non-fucosylated immunoglobrins. Applicant: Yusuke Mimura Yuka Mimura. The sequence listing filed with the application follows.

SEQUENCE LISTING (2 sequences)

SEQ ID NO: 1 - DNA, 1082 bp, Artificial Sequence
  enzyme
ccatggcccatatgatgaacgacaacgtcgcctggttcaaacaggccaaatacggcatgatgatccactggggtctgtatagtctgctggctggcgaatatcgcggtgaaagtagtagcgcatacgcagaatggattcagagcaaattccagatcccgaacgcagaatacggcaatctggcgaccgcgtttaatccgctgtacttcgacgcgaaaaagattgtcgctctggctaaacagtgcggtatgcagtacctggttgttaccaccaaacatcacgacggctttgcgatgtaccatagcaaagtcgacgcgtataacgtctacgacgcaaccccgtttcaccgcgatattattggcgaactggctgaagcttgccagaaagctggtctgaaatttggcctgtactacagccaggatctggattggcacgatccgaatggcggcggttataaaagtaacgacgtcgaaaccgcaggtaccacctgggataatagttgggatttcccggacgaagaccagaaaaacttcgacctgtgcttcgacaacaaaatcctgccgcagatcaaagagatcatgagcaactacggcgatattgcgaccgcttggtttgatgttccgatgaccctgtctgaagcacagagtcagaccatctacgataccgttcgcgaactgcaaccgaactgtctgattaacagccgtctgggcaacggcaaatacgatttcgttagcctgggcgacaacgagatcccgaaaaacaaagaggacatgaacaaaaccgacgtcgactacaacgaaatcaccggctttaaaccgagtccgctgggtctgtacgaaaccgcaggtaccattaacgatagctggggtttctcctatcacgatcagaactggaaaaccccgcgtaccctgtatcgttacaaacagcacctgaacgacttcgggatcaactacctgctgaacgtaggtctggacccgctgggtcgcgttccgatgatggctgaagaaaatctgctggcagcgaaagctctggaagatgaagcaaatcgtgcggccgcactcgagcaccaccaccaccaccactga

SEQ ID NO: 2 - DNA, 2924 bp, Artificial Sequence
  enzyme
catatggaagagaagacagttcaggttcagaagggcctgccgagcatcgacagtctgcattacttaagtgagaatagcaagaaagaattcaaagaggaactgagtaaggcaggtcaggaaagccagaaagttaaggagattctggcaaaagcccagcaggccgataaacaggcacaggaattagccaagatgaagatcccggagaagattccgatgaaaccgttacacggcccgctgtatggtggctattttcgcacctggcatgacaaaaccagcgacccgaccgagaaagacaaggtgaatagcatgggtgaactgccgaaagaggtggatctggccttcatcttccacgactggaccaaggattacagtctgttctggaaagaattagccacaaaacacgttccgaaattaaacaagcagggcacccgtgtgattcgcacaattccttggcgtttcctggccggcggcgataacagcggtattgccgaagataccagcaagtatcctaacaccccggagggcaataaggcactggccaaagccattgttgacgagtacgtgtacaagtacaacctggatggcctggacgttcaggtggaacacgatagcattccgaaagtggacaaaaaagaagacaccgccggcgttgaacgcagcatccaggtttttgaggaaatcggcaagctgatcggtccgaaaggcgttgacaagagccgcctgttcatcatggatagcacctacatggccgacaagaatccgttaatcgaacgtggcgccccttacattaacctgctgttagttcaggtgtacggcagtcagggtgaaaagggcggttgggaaccggttagcaaccgcccggagaagaccatggaggaacgttggcagggttatagcaagtacatccgcccggagcagtacatgattggcttcagcttctatgaggaaaacgcccaggaaggcaacctgtggtatgatatcaacagccgcaaggatgaagacaaggcaaatggcattaatacagatattaccggcacacgcgccgaacgctatgcacgttggcaaccgaagacaggtggcgtgaaaggcggtatcttcagctacgcaatcgaccgtgatggcgtggcccatcagccgaagaaatatgccaaacagaaggagtttaaggacgccacagacaacatcttccatagcgactatagcgttagcaaggccctgaagacagttatgctgaaggacaaaagctatgatctgattgatgaaaaagactttccggacaaggccctgcgcgaagcagttatggcccaggttggcacccgtaaaggcgacctggaacgcttcaatggtacactgcgcctggataatccggccattcagagtctggaaggcctgaataaatttaaaaagctggcccagctggatctgatcggtctgagccgcatcacaaagctggaccgtagcgtgctgcctgcaaacatgaagccgggcaaagacacactggaaaccgtgctggaaacctataaaaaagacaataaagaagagcctgcaaccattccgcctgttagcctgaaagtgagcggcctgaccggtctgaaggaactggacctgagcggtttcgaccgtgaaaccctggcaggtctggatgcagccacattaacaagtttagaaaaagttgacatcagcggcaataaactggacctggcaccgggcaccgagaaccgccagatcttcgacaccatgctgagcaccatcagcaatcatgttggcagcaatgaacagaccgtgaaatttgacaaacagaagccgaccggccactatccggacacctacggcaaaacaagcctgcgcctgcctgtggccaacgaaaaagtggatctgcagagccagctgctgttcggtaccgttaccaaccagggtaccctgatcaatagtgaagcagactataaagcataccagaatcataagatcgccggccgtagctttgtggatagcaactatcactacaacaatttcaaggtgagctatgaaaactacacggttaaagtgaccgatagcacactgggtaccacaaccgataaaacactggccaccgataaagaggagacatacaaagtggacttctttagcccggccgacaaaaccaaagcagtgcacaccgccaaagttattgtgggtgacgaaaaaaccatgatggtgaatttagccgagggcgccacagtgatcggtggcagtgccgatcctgtgaatgcccgtaaggtgtttgatggtcagctgggcagtgaaacagacaacattagcctgggttgggatagcaagcagagcattatctttaaactgaaggaagatggtttaatcaagcactggcgctttttcaatgacagcgcccgtaaccctgaaacaaccaacaagccgatccaagaggcgagtctgcagatcttcaatattaaggactacaacctggacaatttactggaaaatccgaacaaattcgatgatgagaagtactggattaccgtggatacctatagtgcccagggcgagcgcgcaacagcctttagtaacacactgaataatatcaccagcaaatattggcgcgtggtgttcgacacaaaaggcgaccgctatagtagcccggtggttccggaattacaaatcctgggctacccgctgccgaacgcagacaccattatgaagaccgtgaccaccgccaaagaactgagtcagcagaaggataagtttagccagaaaatgctggatgaactgaaaatcaaagaaatggcactggaaacaagtctgaatagcaaaatttttgatgtgacagccatcaacgccaatgcaggcgttctgaaagactgtattgaaaagcgccagctgctgaagaaacatcatcatcatcatcatcatcaccaccactaagcggccgc